European Patent Specification EP 4 071 477 B1, published January 21, 2026. Title: COMPOSITIONS AND METHODS FOR DIAGNOSING LYME DISEASE AND FOR PREDICTING LYME DISEASE SPIROCHETE ELIMINATION AFTER TREATMENT. Applicant: Qiagen Sciences LLC Biopeptides Corp. Gundersen Lutheran Medical Foundation, Inc. The sequence listing filed with the application follows.

SEQUENCE LISTING (40 sequences)

SEQ ID NO: 1 - protein, 25 aa, Borrelia sp.
NVRTAEELGMQPAKINTPASLSGSQ

SEQ ID NO: 2 - protein, 20 aa, Borrelia sp.
NTPASLSGSQASWTLRVHVG

SEQ ID NO: 3 - protein, 20 aa, Borrelia sp.
LSGSQASWTLRVHVGANQDE

SEQ ID NO: 4 - protein, 20 aa, Borrelia sp.
QDEAIAVNIYAANVANLFSG

SEQ ID NO: 5 - protein, 19 aa, Borrelia sp.
SLAKIENAIRMISDQRANL

SEQ ID NO: 6 - protein, 20 aa, Borrelia sp.
SIVMVLFFDLLVACSIGLVE

SEQ ID NO: 7 - protein, 20 aa, Borrelia sp.
LFFDLLVACSIGLVERTNAA

SEQ ID NO: 8 - protein, 25 aa, Borrelia sp.
IGLVERTNAALESSSKDLKNKILKI

SEQ ID NO: 9 - protein, 25 aa, Borrelia sp.
KDLKNKILKIKKEATGKGVLFEAFT

SEQ ID NO: 10 - protein, 25 aa, Borrelia sp.
GKGVLFEAFTGLKTGSKVTSGGLAL

SEQ ID NO: 11 - protein, 25 aa, Borrelia sp.
SKVTSGGLALREAKVQAIVETGKFL

SEQ ID NO: 12 - protein, 25 aa, Borrelia sp.
QAIVETGKFLKIIEEEALKLKETGN

SEQ ID NO: 13 - protein, 25 aa, Borrelia sp.
EALKLKETGNSGQFLAMFDLMLEVV

SEQ ID NO: 14 - protein, 25 aa, Borrelia sp.
AMFDLMLEVVESLEDVGIIGLKARV

SEQ ID NO: 15 - protein, 25 aa, Borrelia sp.
VGIIGLKARVLEESKNNPINTAERL

SEQ ID NO: 16 - protein, 25 aa, Borrelia sp.
NNPINTAERLLAAKAQIENQLKVVK

SEQ ID NO: 17 - protein, 25 aa, Borrelia sp.
QIENQLKVVKEKQNIENGGEKKNNK

SEQ ID NO: 18 - protein, 25 aa, Borrelia sp.
LKVVKEKQNIENGGEKKNNKSKKKK

SEQ ID NO: 19 - protein, 25 aa, Borrelia sp.
FGLSGAYGNETFNNSSITYSLKDKS

SEQ ID NO: 20 - protein, 25 aa, Borrelia sp.
SITYSLKDKSVVGNDLLSPTLSNSA

SEQ ID NO: 21 - protein, 25 aa, Borrelia sp.
LLSPTLSNSAILASFGAKYKLGLTK

SEQ ID NO: 22 - protein, 20 aa, Borrelia sp.
GAKYKLGLTKINDKNTYLIL

SEQ ID NO: 23 - protein, 20 aa, Borrelia sp.
LGLTKINDKNTYLILQMGTD

SEQ ID NO: 24 - protein, 20 aa, Borrelia sp.
TYLILQMGTDFGIDPFASDF

SEQ ID NO: 25 - protein, 20 aa, Borrelia sp.
QMGTDFGIDPFASDFSIFGH

SEQ ID NO: 26 - protein, 25 aa, Borrelia sp.
FASDFSIFGHISKAANFKKETPSDP

SEQ ID NO: 27 - protein, 25 aa, Borrelia sp.
NFKKETPSDPNKKAEIFDPNGNALN

SEQ ID NO: 28 - protein, 25 aa, Borrelia sp.
IFDPNGNALNFSKNTELGIAFSTGA

SEQ ID NO: 29 - protein, 20 aa, Borrelia sp.
ELGIAFSTGASIGFAWNKDT

SEQ ID NO: 30 - protein, 20 aa, Borrelia sp.
FSTGASIGFAWNKDTGEKES

SEQ ID NO: 31 - protein, 25 aa, Borrelia sp.
FSTGASIGFAWNKDTGEKESWAIKG

SEQ ID NO: 32 - protein, 15 aa, Borrelia sp.
KEMLANSVKELTSPI

SEQ ID NO: 33 - protein, 21 aa, Borrelia sp.
ATKAIGKKIQQNGGLAVEAGH

SEQ ID NO: 34 - protein, 40 aa, Borrelia burgdorferi
NVRTAEELGMQPAKINTPASLSGSQASWTLRVHVGANQDE

SEQ ID NO: 35 - protein, 20 aa, Borrelia  burgdorferi
QDEAIAVNIYAANVANLFSG

SEQ ID NO: 36 - protein, 19 aa, Borrelia  burgdorferi
SLAKIENAIRMISDQRANL

SEQ ID NO: 37 - protein, 180 aa, Borrelia burgdorferi
SIVMVLFFDLLVACSIGLVERTNAALESSSKDLKNKILKIKKEATGKGVLFEAFTGLKTGSKVTSGGLALREAKVQAIVETGKFLKIIEEEALKLKETGNSGQFLAMFDLMLEVVESLEDVGIIGLKARVLEESKNNPINTAERLLAAKAQIENQLKVVKEKQNIENGGEKKNNKSKKKK

SEQ ID NO: 38 - protein, 150 aa, Borrelia burgdorferi
FGLSGAYGNETFNNSSITYSLKDKSVVGNDLLSPTLSNSAILASFGAKYKLGLTKINDKNTYLILQMGTDFGIDPFASDFSIFGHISKAANFKKETPSDPNKKAEIFDPNGNALNFSKNTELGIAFSTGASIGFAWNKDTGEKESWAIKG

SEQ ID NO: 39 - protein, 21 aa, Borrelia burgdorferi
ATKAIGKKIQQNGGLAVEAGH

SEQ ID NO: 40 - protein, 15 aa, Borrelia burgdorferi
KEMLANSVKELTSPI